European Patent Application EP 4 223 775 A1, published August 9, 2023. Title: HUMANIZED ANTI-CD22 RECOMBINANT IMMUNOTOXIN AND APPLICATION THEREOF. Applicant: KUNMING SINOWAY NATURAL PHARMACEUTICALS CO., LTD. The sequence listing filed with the application follows.

SEQUENCE LISTING (33 sequences)

SEQ ID NO: 1 - protein, 352 aa, artificial
  PE38 polypeptide sequence
KASGGPEGGSLAALTAHQACHLPLETFTRHRQPRGWEQLEQCGYPVQRLVALYLAARLSWNQVDQVIRNALASPGSGGDLGEAIREQPEQARLALTLAAAESERFVRQGTGNDEAGAANGPADSGDALLERNYPTGAEFLGDGGDVSFSTRGTQNWTVERLLQAHRQLEERGYVFVGYHGTFLEAAQSIVFGGVRARSQDLDAIWRGFYIAGDPALAYGYAQDQEPDARGRIRNGALLRVYVPRSSLPGFYRTSLTLAAPEAAGEVERLIGHPLPLRLDAITGPEEEGGRLETILGWPLAERTVVIPSAIPTDPRNVGGDLDPSSIPDKEQAISALPDYASQPGKPPREDLK

SEQ ID NO: 2 - protein, 124 aa, artificial
  HA22, VH polypeptide sequence
MEVQLVESGGGLVKPGGSLKLSCAASGFAFSIYDMSWVRQTPEKCLEWVAYISSGGGTTYYPDTVKGRFTISRDNAKNTLYLQMSSLKSEDTAMYYCARHSGYGTHWGVLFAYWGQGTLVTVSA

SEQ ID NO: 3 - protein, 124 aa, artificial
  Version 1 VH polypeptide sequence
MEVQLVESGGGLVKPGGSLRLSCAASGFAFSIYDMSWVRQAPGKCLEWVAYISSGGGTTYYPDSVKGRFTISRENAKNSLYLQMNSLKSEDTAMYYCARHSGYGTHWGVLFAYWGQGTMVTVSS

SEQ ID NO: 4 - protein, 124 aa, artificial
  Version 2 VH polypeptide sequence
MEVQLVESGGGLVKPGGSLRLSCAASGFAFSIYDMSWVRQTPEKCLEWVAYISSGGGTTYYPDSVKGRFTISRENAKNSLYLQMNSLKSEDTAMYYCARHSGYGTHWGVLFAYWGQGTMVTVSS

SEQ ID NO: 5 - protein, 124 aa, artificial
  Version 3 VH polypeptide sequence
MEVQLVESGGGLVKPGGSLRLSCAASGFAFSIYDMSWIRQAPGKCLEWVSYISSGGGTTYYPGSVKGRFTISRENAKNSLYLQMNSLRAGDTAVYYCARHSGYGTHWGVLFAYWGQGTMVTVSS

SEQ ID NO: 6 - protein, 124 aa, artificial
  Version 4 VH polypeptide sequence
MEVQLVESGGGLVKPGGSLRLSCAASGFAFSIYDMSWIRQAPGKCLEWVAYISSGGGTTYYPGSVKGRFTISRENAKNSLYLQMNSLRAGDTAVYYCARHSGYGTHWGVLFAYWGQGTMVTVSS

SEQ ID NO: 7 - protein, 124 aa, artificial
  Version 5 VH polypeptide sequence
MEVQLVESGGGLVKPGGSLRLSCAASGFAFSIYDMSWIRQAPGKCLEWVAYISSGGGTTYYPGSVKGRFTISRENAKNSLYLQMNSLRSEDTAVYYCARHSGYGTHWGVLFAYWGQGTMVTVSS

SEQ ID NO: 8 - protein, 476 aa, artificial
  HA22 VH-PE38 polypeptide sequence
MEVQLVESGGGLVKPGGSLKLSCAASGFAFSIYDMSWVRQTPEKCLEWVAYISSGGGTTYYPDTVKGRFTISRDNAKNTLYLQMSSLKSEDTAMYYCARHSGYGTHWGVLFAYWGQGTLVTVSAKASGGPEGGSLAALTAHQACHLPLETFTRHRQPRGWEQLEQCGYPVQRLVALYLAARLSWNQVDQVIRNALASPGSGGDLGEAIREQPEQARLALTLAAAESERFVRQGTGNDEAGAANGPADSGDALLERNYPTGAEFLGDGGDVSFSTRGTQNWTVERLLQAHRQLEERGYVFVGYHGTFLEAAQSIVFGGVRARSQDLDAIWRGFYIAGDPALAYGYAQDQEPDARGRIRNGALLRVYVPRSSLPGFYRTSLTLAAPEAAGEVERLIGHPLPLRLDAITGPEEEGGRLETILGWPLAERTVVIPSAIPTDPRNVGGDLDPSSIPDKEQAISALPDYASQPGKPPREDLK

SEQ ID NO: 9 - protein, 476 aa, artificial
  Version 1 VH-PE38 polypeptide sequence
MEVQLVESGGGLVKPGGSLRLSCAASGFAFSIYDMSWVRQAPGKCLEWVAYISSGGGTTYYPDSVKGRFTISRENAKNSLYLQMNSLKSEDTAMYYCARHSGYGTHWGVLFAYWGQGTMVTVSSKASGGPEGGSLAALTAHQACHLPLETFTRHRQPRGWEQLEQCGYPVQRLVALYLAARLSWNQVDQVIRNALASPGSGGDLGEAIREQPEQARLALTLAAAESERFVRQGTGNDEAGAANGPADSGDALLERNYPTGAEFLGDGGDVSFSTRGTQNWTVERLLQAHRQLEERGYVFVGYHGTFLEAAQSIVFGGVRARSQDLDAIWRGFYIAGDPALAYGYAQDQEPDARGRIRNGALLRVYVPRSSLPGFYRTSLTLAAPEAAGEVERLIGHPLPLRLDAITGPEEEGGRLETILGWPLAERTVVIPSAIPTDPRNVGGDLDPSSIPDKEQAISALPDYASQPGKPPREDLK

SEQ ID NO: 10 - protein, 476 aa, artificial
  Version 2 VH-PE38 polypeptide sequence
MEVQLVESGGGLVKPGGSLRLSCAASGFAFSIYDMSWVRQTPEKCLEWVAYISSGGGTTYYPDSVKGRFTISRENAKNSLYLQMNSLKSEDTAMYYCARHSGYGTHWGVLFAYWGQGTMVTVSSKASGGPEGGSLAALTAHQACHLPLETFTRHRQPRGWEQLEQCGYPVQRLVALYLAARLSWNQVDQVIRNALASPGSGGDLGEAIREQPEQARLALTLAAAESERFVRQGTGNDEAGAANGPADSGDALLERNYPTGAEFLGDGGDVSFSTRGTQNWTVERLLQAHRQLEERGYVFVGYHGTFLEAAQSIVFGGVRARSQDLDAIWRGFYIAGDPALAYGYAQDQEPDARGRIRNGALLRVYVPRSSLPGFYRTSLTLAAPEAAGEVERLIGHPLPLRLDAITGPEEEGGRLETILGWPLAERTVVIPSAIPTDPRNVGGDLDPSSIPDKEQAISALPDYASQPGKPPREDLK

SEQ ID NO: 11 - protein, 476 aa, artificial
  Version 3 VH-PE38 polypeptide sequence
MEVQLVESGGGLVKPGGSLRLSCAASGFAFSIYDMSWIRQAPGKCLEWVSYISSGGGTTYYPGSVKGRFTISRENAKNSLYLQMNSLRAGDTAVYYCARHSGYGTHWGVLFAYWGQGTMVTVSSKASGGPEGGSLAALTAHQACHLPLETFTRHRQPRGWEQLEQCGYPVQRLVALYLAARLSWNQVDQVIRNALASPGSGGDLGEAIREQPEQARLALTLAAAESERFVRQGTGNDEAGAANGPADSGDALLERNYPTGAEFLGDGGDVSFSTRGTQNWTVERLLQAHRQLEERGYVFVGYHGTFLEAAQSIVFGGVRARSQDLDAIWRGFYIAGDPALAYGYAQDQEPDARGRIRNGALLRVYVPRSSLPGFYRTSLTLAAPEAAGEVERLIGHPLPLRLDAITGPEEEGGRLETILGWPLAERTVVIPSAIPTDPRNVGGDLDPSSIPDKEQAISALPDYASQPGKPPREDLK

SEQ ID NO: 12 - protein, 476 aa, artificial
  Version 4 VH-PE38 polypeptide sequence
MEVQLVESGGGLVKPGGSLRLSCAASGFAFSIYDMSWIRQAPGKCLEWVAYISSGGGTTYYPGSVKGRFTISRENAKNSLYLQMNSLRAGDTAVYYCARHSGYGTHWGVLFAYWGQGTMVTVSSKASGGPEGGSLAALTAHQACHLPLETFTRHRQPRGWEQLEQCGYPVQRLVALYLAARLSWNQVDQVIRNALASPGSGGDLGEAIREQPEQARLALTLAAAESERFVRQGTGNDEAGAANGPADSGDALLERNYPTGAEFLGDGGDVSFSTRGTQNWTVERLLQAHRQLEERGYVFVGYHGTFLEAAQSIVFGGVRARSQDLDAIWRGFYIAGDPALAYGYAQDQEPDARGRIRNGALLRVYVPRSSLPGFYRTSLTLAAPEAAGEVERLIGHPLPLRLDAITGPEEEGGRLETILGWPLAERTVVIPSAIPTDPRNVGGDLDPSSIPDKEQAISALPDYASQPGKPPREDLK

SEQ ID NO: 13 - protein, 476 aa, artificial
  Version 5 VH-PE38 polypeptide sequence
MEVQLVESGGGLVKPGGSLRLSCAASGFAFSIYDMSWIRQAPGKCLEWVAYISSGGGTTYYPGSVKGRFTISRENAKNSLYLQMNSLRSEDTAVYYCARHSGYGTHWGVLFAYWGQGTMVTVSSKASGGPEGGSLAALTAHQACHLPLETFTRHRQPRGWEQLEQCGYPVQRLVALYLAARLSWNQVDQVIRNALASPGSGGDLGEAIREQPEQARLALTLAAAESERFVRQGTGNDEAGAANGPADSGDALLERNYPTGAEFLGDGGDVSFSTRGTQNWTVERLLQAHRQLEERGYVFVGYHGTFLEAAQSIVFGGVRARSQDLDAIWRGFYIAGDPALAYGYAQDQEPDARGRIRNGALLRVYVPRSSLPGFYRTSLTLAAPEAAGEVERLIGHPLPLRLDAITGPEEEGGRLETILGWPLAERTVVIPSAIPTDPRNVGGDLDPSSIPDKEQAISALPDYASQPGKPPREDLK

SEQ ID NO: 14 - protein, 108 aa, artificial
  HA22, VL polypeptide sequence
MDIQMTQTTSSLSASLGDRVTISCRASQDISNYLNWYQQKPDGTVKLLIYYTSILHSGVPSRFSGSGSGTDYSLTISNLEQEDFATYFCQQGNTLPWTFGCGTKLEIK

SEQ ID NO: 15 - protein, 108 aa, artificial
  Version 1 VL polypeptide sequence
MDIQMTQSPSTLSASVGDRVTITCRASQDISNYLNWYQQRPGQSVKLLIYYTSILHSGVPSRFSGSGSGTDYTLTISSLQPEDFATYFCQQGNTLPWTFGCGTKVEIK

SEQ ID NO: 16 - protein, 108 aa, artificial
  Version 2 VL polypeptide sequence
MDIQMTQSTSTLSASVGDRVTITCRASQDISNYLNWYQQRPDGSVKLLIYYTSILHSGVPSRFSGSGSGTDYTLTISSLQDEDFATYFCQQGNTLPWTFGCGTKVEIK

SEQ ID NO: 17 - protein, 108 aa, artificial
  Version 3 VL polypeptide sequence
MDIQMTQSPSTLSASVGDRVTITCRASQDISNYLNWFQQRPGQSPRRLIYYTSILHSGVPSRFSGSGSGTDYTLTISSLQPEDFATYYCQQGNTLPWTFGCGTKVEIK

SEQ ID NO: 18 - protein, 108 aa, artificial
  Version 4 VL polypeptide sequence
MDIQMTQSPSTLSASVGDRVTITCRASQDISNYLNWFQQRPGQSPRLLIYYTSILHSGVPSRFSGSGSGTDYTLTISSLQPEDFATYYCQQGNTLPWTFGCGTKVEIK

SEQ ID NO: 19 - DNA, 1428 bp, artificial
  Version 1 VH-PE38 DNA sequence
atggaagtgcagctggtggaatccggcggaggcctggtcaagcccggcggctctctgagactgtcctgcgctgcttctggcttcgccttctccatctacgacatgtcctgggtcagacaggcccctggcaagtgcctggaatgggtggcctacatctcctctggcggaggcaccacctactaccctgactccgtgaagggcagattcaccatctctagagagaacgccaagaacagcctgtacctgcagatgaactccctgaagtccgaggacaccgccatgtactactgcgccagacactccggctacggcacacactggggcgtgctgttcgcttactggggccagggcaccatggtgaccgtgtcctccaaagcgtcaggcggtccggaaggcggttcgctggcagctctgaccgcacatcaggcatgccacctgccgctggaaacctttacccgccatcgtcaaccgcgcggctgggaacagctggaacaatgtggttatccggtgcagcgcctggttgccctgtacctggccgcacgtctgagctggaaccaggttgatcaagtcattcgtaatgcgctggcatcaccgggctcgggcggtgacctgggtgaagcaatccgcgaacagccggaacaagcgcgcctggccctgaccctggcagctgcggaatccgaacgctttgtgcgtcagggcaccggtaatgatgaagccggtgcagcaaatggtccggctgattcaggtgacgcgctgctggaacgcaactatccgacgggcgccgaatttctgggtgatggcggtgacgtgagtttctccacccgcggcacgcagaattggaccgttgaacgtctgctgcaggcgcatcgccaactggaagaacgtggttatgtttttgtcggctatcatggcacctttctggaagctgcgcagtcgattgtctttggcggtgtgcgtgcacgcagccaggatctggatgcaatttggcgcggcttctacatcgcaggtgatccggctctggcgtatggctacgctcaggatcaagaaccggatgcgcgtggccgcatccgtaatggtgccctgctgcgtgtgtatgttccgcgttcatcgctgccgggtttttaccgtacctctctgaccctggcggcaccggaagctgccggcgaagtggaacgcctgattggtcacccgctgccgctgcgtctggatgcaatcaccggtccggaagaagaaggcggccgtctggaaacgattctgggttggccgctggccgaacgtaccgtggttattccgagcgcaatcccgacggacccgcgcaatgttggcggtgatctggacccgagctctattccggataaagaacaggccatctccgcactgccggactatgcgtcacaaccgggcaaaccgccgcgtgaagacctgaaa

SEQ ID NO: 20 - DNA, 1428 bp, artificial
  Version 2 VH-PE38 DNA sequence
atggaagtgcagctggtggaatccggcggaggcctggtcaagcccggcggctctctgagactgtcctgcgctgcttctggcttcgccttctccatctacgacatgtcctgggtcagacagacccctgaaaagtgcctggaatgggtggcctacatctcctctggcggaggcaccacctactaccctgactccgtgaagggcagattcaccatctctagagagaacgccaagaacagcctgtacctgcagatgaactccctgaagtccgaggacaccgccatgtactactgcgccagacactccggctacggcacacactggggcgtgctgttcgcttactggggccagggcaccatggtgaccgtgtcctccaaagcgtcaggcggtccggaaggcggttcgctggcagctctgaccgcacatcaggcatgccacctgccgctggaaacctttacccgccatcgtcaaccgcgcggctgggaacagctggaacaatgtggttatccggtgcagcgcctggttgccctgtacctggccgcacgtctgagctggaaccaggttgatcaagtcattcgtaatgcgctggcatcaccgggctcgggcggtgacctgggtgaagcaatccgcgaacagccggaacaagcgcgcctggccctgaccctggcagctgcggaatccgaacgctttgtgcgtcagggcaccggtaatgatgaagccggtgcagcaaatggtccggctgattcaggtgacgcgctgctggaacgcaactatccgacgggcgccgaatttctgggtgatggcggtgacgtgagtttctccacccgcggcacgcagaattggaccgttgaacgtctgctgcaggcgcatcgccaactggaagaacgtggttatgtttttgtcggctatcatggcacctttctggaagctgcgcagtcgattgtctttggcggtgtgcgtgcacgcagccaggatctggatgcaatttggcgcggcttctacatcgcaggtgatccggctctggcgtatggctacgctcaggatcaagaaccggatgcgcgtggccgcatccgtaatggtgccctgctgcgtgtgtatgttccgcgttcatcgctgccgggtttttaccgtacctctctgaccctggcggcaccggaagctgccggcgaagtggaacgcctgattggtcacccgctgccgctgcgtctggatgcaatcaccggtccggaagaagaaggcggccgtctggaaacgattctgggttggccgctggccgaacgtaccgtggttattccgagcgcaatcccgacggacccgcgcaatgttggcggtgatctggacccgagctctattccggataaagaacaggccatctccgcactgccggactatgcgtcacaaccgggcaaaccgccgcgtgaagacctgaaa

SEQ ID NO: 21 - DNA, 1428 bp, artificial
  Version 3 VH-PE38 DNA sequence
atggaagtgcagctggttgaaagcggtggcggtctggtgaaaccgggcggtagcctgcgtctgagctgcgcggcgagcggtttcgcgtttagcatctacgacatgagctggattcgtcaagcgccgggcaaatgcctggagtgggtgagctatatcagcagcggcggtggcaccacctactatccgggtagcgttaagggccgtttcaccattagccgtgaaaacgcgaaaaacagcctgtacctgcagatgaacagcctgcgtgcgggtgataccgctgtgtactattgcgcgcgtcacagcggttacggcacccactggggcgttctgtttgcgtattggggtcaaggcaccatggtgaccgttagcagcaaagcgtcaggcggtccggaaggcggttcgctggcagctctgaccgcacatcaggcatgccacctgccgctggaaacctttacccgccatcgtcaaccgcgcggctgggaacagctggaacaatgtggttatccggtgcagcgcctggttgccctgtacctggccgcacgtctgagctggaaccaggttgatcaagtcattcgtaatgcgctggcatcaccgggctcgggcggtgacctgggtgaagcaatccgcgaacagccggaacaagcgcgcctggccctgaccctggcagctgcggaatccgaacgctttgtgcgtcagggcaccggtaatgatgaagccggtgcagcaaatggtccggctgattcaggtgacgcgctgctggaacgcaactatccgacgggcgccgaatttctgggtgatggcggtgacgtgagtttctccacccgcggcacgcagaattggaccgttgaacgtctgctgcaggcgcatcgccaactggaagaacgtggttatgtttttgtcggctatcatggcacctttctggaagctgcgcagtcgattgtctttggcggtgtgcgtgcacgcagccaggatctggatgcaatttggcgcggcttctacatcgcaggtgatccggctctggcgtatggctacgctcaggatcaagaaccggatgcgcgtggccgcatccgtaatggtgccctgctgcgtgtgtatgttccgcgttcatcgctgccgggtttttaccgtacctctctgaccctggcggcaccggaagctgccggcgaagtggaacgcctgattggtcacccgctgccgctgcgtctggatgcaatcaccggtccggaagaagaaggcggccgtctggaaacgattctgggttggccgctggccgaacgtaccgtggttattccgagcgcaatcccgacggacccgcgcaatgttggcggtgatctggacccgagctctattccggataaagaacaggccatctccgcactgccggactatgcgtcacaaccgggcaaaccgccgcgtgaagacctgaaa

SEQ ID NO: 22 - DNA, 1428 bp, artificial
  Version 4 VH-PE38 DNA sequence
atggaagtgcagctggttgaaagcggtggcggtctggtgaaaccgggcggtagcctgcgtctgagctgcgcggcgagcggtttcgcgtttagcatctacgacatgagctggattcgtcaagcgccgggcaaatgcctggagtgggtggcgtatatcagcagcggcggtggcaccacctactatccgggtagcgttaagggccgtttcaccattagccgtgaaaacgcgaaaaacagcctgtacctgcagatgaacagcctgcgtgcgggtgataccgctgtgtactattgcgcgcgtcacagcggttacggcacccactggggcgttctgtttgcgtattggggtcaaggcaccatggtgaccgttagcagcaaagcgtcaggcggtccggaaggcggttcgctggcagctctgaccgcacatcaggcatgccacctgccgctggaaacctttacccgccatcgtcaaccgcgcggctgggaacagctggaacaatgtggttatccggtgcagcgcctggttgccctgtacctggccgcacgtctgagctggaaccaggttgatcaagtcattcgtaatgcgctggcatcaccgggctcgggcggtgacctgggtgaagcaatccgcgaacagccggaacaagcgcgcctggccctgaccctggcagctgcggaatccgaacgctttgtgcgtcagggcaccggtaatgatgaagccggtgcagcaaatggtccggctgattcaggtgacgcgctgctggaacgcaactatccgacgggcgccgaatttctgggtgatggcggtgacgtgagtttctccacccgcggcacgcagaattggaccgttgaacgtctgctgcaggcgcatcgccaactggaagaacgtggttatgtttttgtcggctatcatggcacctttctggaagctgcgcagtcgattgtctttggcggtgtgcgtgcacgcagccaggatctggatgcaatttggcgcggcttctacatcgcaggtgatccggctctggcgtatggctacgctcaggatcaagaaccggatgcgcgtggccgcatccgtaatggtgccctgctgcgtgtgtatgttccgcgttcatcgctgccgggtttttaccgtacctctctgaccctggcggcaccggaagctgccggcgaagtggaacgcctgattggtcacccgctgccgctgcgtctggatgcaatcaccggtccggaagaagaaggcggccgtctggaaacgattctgggttggccgctggccgaacgtaccgtggttattccgagcgcaatcccgacggacccgcgcaatgttggcggtgatctggacccgagctctattccggataaagaacaggccatctccgcactgccggactatgcgtcacaaccgggcaaaccgccgcgtgaagacctgaaa

SEQ ID NO: 23 - DNA, 1428 bp, artificial
  Version 5 VH-PE38 DNA sequence
atggaagtgcagctggttgaaagcggtggcggtctggtgaaaccgggcggtagcctgcgtctgagctgcgcggcgagcggtttcgcgtttagcatctacgacatgagctggattcgtcaagcgccgggcaaatgcctggagtgggtggcgtatatcagcagcggcggtggcaccacctactatccgggtagcgttaagggccgtttcaccattagccgtgaaaacgcgaaaaacagcctgtacctgcagatgaacagcctgcgttctgaggataccgctgtgtactattgcgcgcgtcacagcggttacggcacccactggggcgttctgtttgcgtattggggtcaaggcaccatggtgaccgttagcagcaaagcgtcaggcggtccggaaggcggttcgctggcagctctgaccgcacatcaggcatgccacctgccgctggaaacctttacccgccatcgtcaaccgcgcggctgggaacagctggaacaatgtggttatccggtgcagcgcctggttgccctgtacctggccgcacgtctgagctggaaccaggttgatcaagtcattcgtaatgcgctggcatcaccgggctcgggcggtgacctgggtgaagcaatccgcgaacagccggaacaagcgcgcctggccctgaccctggcagctgcggaatccgaacgctttgtgcgtcagggcaccggtaatgatgaagccggtgcagcaaatggtccggctgattcaggtgacgcgctgctggaacgcaactatccgacgggcgccgaatttctgggtgatggcggtgacgtgagtttctccacccgcggcacgcagaattggaccgttgaacgtctgctgcaggcgcatcgccaactggaagaacgtggttatgtttttgtcggctatcatggcacctttctggaagctgcgcagtcgattgtctttggcggtgtgcgtgcacgcagccaggatctggatgcaatttggcgcggcttctacatcgcaggtgatccggctctggcgtatggctacgctcaggatcaagaaccggatgcgcgtggccgcatccgtaatggtgccctgctgcgtgtgtatgttccgcgttcatcgctgccgggtttttaccgtacctctctgaccctggcggcaccggaagctgccggcgaagtggaacgcctgattggtcacccgctgccgctgcgtctggatgcaatcaccggtccggaagaagaaggcggccgtctggaaacgattctgggttggccgctggccgaacgtaccgtggttattccgagcgcaatcccgacggacccgcgcaatgttggcggtgatctggacccgagctctattccggataaagaacaggccatctccgcactgccggactatgcgtcacaaccgggcaaaccgccgcgtgaagacctgaaa

SEQ ID NO: 24 - DNA, 324 bp, artificial
  Version 1 VL DNA sequence
atggacatccagatgacccagtctccttctacactgtctgcttctgtgggcgacagagtgaccatcacctgcagagcctctcaggacatctccaactacctgaactggtaccagcagagacctggccagtccgtgaagctgctgatctactacacctccatcctgcactccggcgtgccttccagattctccggctctggatctggcaccgactacaccctgaccatctcctccctgcagcctgaggacttcgccacctacttctgccagcagggcaacaccctgccttggaccttcggctgcggcaccaaggtggaaatcaag

SEQ ID NO: 25 - DNA, 324 bp, artificial
  Version 2 VL DNA sequence
atggacatccagatgacccagtctacttctacactgtctgcttctgtgggcgacagagtgaccatcacctgcagagcctctcaggacatctccaactacctgaactggtaccagcagagacctgatggctccgtgaagctgctgatctactacacctccatcctgcactccggcgtgccttccagattctccggctctggatctggcaccgactacaccctgaccatctcctccctgcaggatgaggacttcgccacctacttctgccagcagggcaacaccctgccttggaccttcggctgcggcaccaaggtggaaatcaag

SEQ ID NO: 26 - DNA, 324 bp, artificial
  Version 3 VL DNA sequence
atggacatccagatgacccagagcccgagcaccctgagcgcgagcgtgggcgaccgtgttaccatcacctgccgtgcgagccaggatattagcaactacctgaactggtttcaacaacgtccgggtcaaagcccgcgtcgtctgatctactataccagcattctgcacagcggtgtgccgagccgttttagcggtagcggcagcggtaccgactataccctgaccatcagcagcctgcagccggaggatttcgcgacctactattgccagcagggtaacaccctgccgtggacctttggctgcggtaccaaggttgaaattaaa

SEQ ID NO: 27 - DNA, 324 bp, artificial
  Version 3 VL DNA sequence
atggacatccagatgacccagagcccgagcaccctgagcgcgagcgtgggcgaccgtgttaccatcacctgccgtgcgagccaggatattagcaactacctgaactggtttcaacaacgtccgggtcaaagcccgcgtctgctgatctactataccagcattctgcacagcggtgtgccgagccgttttagcggtagcggcagcggtaccgactataccctgaccatcagcagcctgcagccggaggatttcgcgacctactattgccagcagggtaacaccctgccgtggacctttggctgcggtaccaaggttgaaattaaa

SEQ ID NO: 28 - protein, 8 aa, artificial
  HA22, H-CDR1
GFAFSIYD

SEQ ID NO: 29 - protein, 9 aa, artificial
  HA22, H-CDR2
ISSGGGTTY

SEQ ID NO: 30 - protein, 17 aa, artificial
  HA22, H-CDR3
CARHSGYGTHWGVLFAY

SEQ ID NO: 31 - protein, 6 aa, artificial
  HA22, L-CDR1
QDISNY

SEQ ID NO: 32 - protein, 8 aa, artificial
  HA22, L-CDR2
YTSILHSG

SEQ ID NO: 33 - protein, 7 aa, artificial
  HA22, L-CDR3
QQGNTLP